European Patent Application EP 4 458 976 A1, published November 6, 2024. Title: RECOMBINANT ADENO-ASSOCIATED VIRUS (RAAV) GENOME AND SINGLE-POLARITY RAAV VECTOR PACKAGED THEREBY. Applicant: SUZHOU GENEHEALTH BIOTECHNOLOGY，CO., LTD. The sequence listing filed with the application follows.

SEQUENCE LISTING (19 sequences)

SEQ ID NO: 1 - DNA, 145 bp, adeno-associated virus type 2
  source 1..145: mol_type = genomic DNA
aggaacccctagtgatggagttggccactccctctctgcgcgctcgctcgctcactgaggccgcccgggcaaagcccgggcgtcgggcgacctttggtcgcccggcctcagtgagcgagcgagcgcgcagagagggagtggccaa

SEQ ID NO: 2 - DNA, 145 bp, adeno-associated virus type 2
  source 1..145: mol_type = genomic DNA
aggaacccctagtgatggagttggccactccctctctgcgcgctcgctcgctcactgaggccgggcgaccaaaggtcgcccgacgcccgggctttgcccgggcggcctcagtgagcgagcgagcgcgcagagagggagtggccaa

SEQ ID NO: 3 - DNA, 16 bp, adeno-associated virus type 2
  source 1..16: mol_type = genomic DNA
gcgcgctcgctcgctc

SEQ ID NO: 4 - skipped

SEQ ID NO: 5 - DNA, 73 bp, adeno-associated virus type 2
  source 1..73: mol_type = other DNA
aggaacccctagtgatggagttggccactccctctctgcgcgctcgctcgctcactgaggccgggcgaccaaa

SEQ ID NO: 6 - DNA, 75 bp, Artificial sequence
  source 1..75: mol_type = unassigned DNA
caggaacccctagtgatggagttggccactccctctctgcgcgctcgctcgctcactgaggccgggcgaccaaaa

SEQ ID NO: 7 - DNA, 83 bp, Artificial sequence
  source 1..83: mol_type = unassigned DNA
cgcgttttggtcgcccggcctcagtgagcgagcgagcgcgcagagagggagtggccaactccatcactaggggttcctggtac

SEQ ID NO: 8 - DNA, 28 bp, Artificial sequence
  source 1..28: mol_type = unassigned DNA
gaccgataatctctagattgaggaacaa

SEQ ID NO: 9 - DNA, 29 bp, Artificial sequence
  source 1..29: mol_type = unassigned DNA
agctttgttcctcaatctagagattatcg

SEQ ID NO: 10 - DNA, 33 bp, Artificial sequence
  source 1..33: mol_type = unassigned DNA
tcactgacgcgtcggaaggtcggtatccacgga

SEQ ID NO: 11 - DNA, 40 bp, Artificial sequence
  source 1..40: mol_type = unassigned DNA
cttcaaccggctgaagctggctagttattaatagtaatca

SEQ ID NO: 12 - DNA, 40 bp, Artificial sequence
  source 1..40: mol_type = unassigned DNA
tgattactattaataactagccagcttcagccggttgaag

SEQ ID NO: 13 - DNA, 33 bp, Artificial sequence
  source 1..33: mol_type = unassigned DNA
cccggggaattcaatcgatgttcgaatcccaat

SEQ ID NO: 14 - DNA, 34 bp, Artificial sequence
  source 1..34: mol_type = unassigned DNA
tttgtaggtaacctcaagaagcacatcctgaatc

SEQ ID NO: 15 - DNA, 34 bp, Artificial sequence
  source 1..34: mol_type = unassigned DNA
gcacgtggttaccttgcccagaatgtctgtgctg

SEQ ID NO: 16 - DNA, 33 bp, Artificial sequence
  source 1..33: mol_type = unassigned DNA
tcactgacgcgtcacgtggttaccttgcccaga

SEQ ID NO: 17 - DNA, 34 bp, Artificial sequence
  source 1..34: mol_type = unassigned DNA
caagatcggtccgcggaaggtcggtatccacgga

SEQ ID NO: 18 - DNA, 21 bp, Artificial sequence
  source 1..21: mol_type = unassigned DNA
tccgcgttacataacttacgg

SEQ ID NO: 19 - DNA, 20 bp, Artificial sequence
  source 1..20: mol_type = unassigned DNA
gggcgtacttggcatatgat